European Patent Application EP 4 524 162 A1, published March 19, 2025. Title: 항-키티나제-3-유사 단백질 1 항체. Applicant: 재단법인 오송첨단의료산업진흥재단. Application KR. The sequence listing filed with the application follows.

SEQUENCE LISTING (160 sequences)

SEQ ID NO: 1 - protein, 11 aa, synthetic construct
  REGION 1..11: note = CDRL1
RASQSISRWLN

SEQ ID NO: 2 - protein, 7 aa, synthetic construct
  REGION 1..7: note = CDRL2
ATSTLQS

SEQ ID NO: 3 - protein, 9 aa, synthetic construct
  REGION 1..9: note = CDRL3
QQSYSFPWT

SEQ ID NO: 4 - protein, 11 aa, synthetic construct
  REGION 1..11: note = CDRL1
RASQDISNYLN

SEQ ID NO: 5 - protein, 7 aa, synthetic construct
  REGION 1..7: note = CDRL2
AASSLQS

SEQ ID NO: 6 - protein, 9 aa, synthetic construct
  REGION 1..9: note = CDRL3
QQSYSFPYT

SEQ ID NO: 7 - protein, 11 aa, synthetic construct
  REGION 1..11: note = CDRL1
RASQSISRYLN

SEQ ID NO: 8 - protein, 7 aa, synthetic construct
  REGION 1..7: note = CDRL2
AASSLQS

SEQ ID NO: 9 - protein, 9 aa, synthetic construct
  REGION 1..9: note = CDRL3
QQSSSTPWT

SEQ ID NO: 10 - protein, 11 aa, synthetic construct
  REGION 1..11: note = CDRL1
RASQDISSWLN

SEQ ID NO: 11 - protein, 7 aa, synthetic construct
  REGION 1..7: note = CDRL2
AASRLQS

SEQ ID NO: 12 - protein, 9 aa, synthetic construct
  REGION 1..9: note = CDRL3
QQAYSFPWT

SEQ ID NO: 13 - protein, 11 aa, synthetic construct
  REGION 1..11: note = CDRL1
RASQSISNWLN

SEQ ID NO: 14 - protein, 7 aa, synthetic construct
  REGION 1..7: note = CDRL2
ATSRLQS

SEQ ID NO: 15 - protein, 9 aa, synthetic construct
  REGION 1..9: note = CDRL3
QQSYSFPYT

SEQ ID NO: 16 - protein, 11 aa, synthetic construct
  REGION 1..11: note = CDRL1
RASQSISRWLN

SEQ ID NO: 17 - protein, 7 aa, synthetic construct
  REGION 1..7: note = CDRL2
AASRLQS

SEQ ID NO: 18 - protein, 9 aa, synthetic construct
  REGION 1..9: note = CDRL3
QQSYSTPWT

SEQ ID NO: 19 - protein, 11 aa, synthetic construct
  REGION 1..11: note = CDRL1
RASQSISNWLN

SEQ ID NO: 20 - protein, 7 aa, synthetic construct
  REGION 1..7: note = CDRL2
ATSRLQS

SEQ ID NO: 21 - protein, 9 aa, synthetic construct
  REGION 1..9: note = CDRL3
QQSYSFPLT

SEQ ID NO: 22 - protein, 11 aa, synthetic construct
  REGION 1..11: note = CDRL1
RASQSISNYLN

SEQ ID NO: 23 - protein, 7 aa, synthetic construct
  REGION 1..7: note = CDRL2
ATSTLHS

SEQ ID NO: 24 - protein, 9 aa, synthetic construct
  REGION 1..9: note = CDRL3
QQSYSFPWT

SEQ ID NO: 25 - protein, 11 aa, synthetic construct
  REGION 1..11: note = CDRL1
RASQDISRWLN

SEQ ID NO: 26 - protein, 7 aa, synthetic construct
  REGION 1..7: note = CDRL2
AASTLQS

SEQ ID NO: 27 - protein, 9 aa, synthetic construct
  REGION 1..9: note = CDRL3
QQSYSFPLT

SEQ ID NO: 28 - protein, 11 aa, synthetic construct
  REGION 1..11: note = CDRL1
RASQSISSWLN

SEQ ID NO: 29 - protein, 7 aa, synthetic construct
  REGION 1..7: note = CDRL2
AASRLQS

SEQ ID NO: 30 - protein, 9 aa, synthetic construct
  REGION 1..9: note = CDRL3
QQTYSFPWT

SEQ ID NO: 31 - protein, 5 aa, synthetic construct
  REGION 1..5: note = CDRH1
SYGMS

SEQ ID NO: 32 - protein, 17 aa, synthetic construct
  REGION 1..17: note = CDRH2
AIKGSGGSTYYADSVKG

SEQ ID NO: 33 - protein, 8 aa, synthetic construct
  REGION 1..8: note = CDRH3
TYGGEIDY

SEQ ID NO: 34 - protein, 5 aa, synthetic construct
  REGION 1..5: note = CDRH1
DYAMS

SEQ ID NO: 35 - protein, 17 aa, synthetic construct
  REGION 1..17: note = CDRH2
GISSSGGTIYYADSVKG

SEQ ID NO: 36 - protein, 8 aa, synthetic construct
  REGION 1..8: note = CDRH3
AIGSWADI

SEQ ID NO: 37 - protein, 5 aa, synthetic construct
  REGION 1..5: note = CDRH1
SYAMH

SEQ ID NO: 38 - protein, 17 aa, synthetic construct
  REGION 1..17: note = CDRH2
AISSSSGTIYYADSVKG

SEQ ID NO: 39 - protein, 8 aa, synthetic construct
  REGION 1..8: note = CDRH3
DFGAVFDY

SEQ ID NO: 40 - protein, 5 aa, synthetic construct
  REGION 1..5: note = CDRH1
SYAMH

SEQ ID NO: 41 - protein, 17 aa, synthetic construct
  REGION 1..17: note = CDRH2
SIKSSGGSKNYADSVKG

SEQ ID NO: 42 - protein, 8 aa, synthetic construct
  REGION 1..8: note = CDRH3
GYGASFDF

SEQ ID NO: 43 - protein, 5 aa, synthetic construct
  REGION 1..5: note = CDRH1
SYAMH

SEQ ID NO: 44 - protein, 17 aa, synthetic construct
  REGION 1..17: note = CDRH2
AISSSGGSIYYADSVKG

SEQ ID NO: 45 - protein, 7 aa, synthetic construct
  REGION 1..7: note = CDRH3
QGLSFDI

SEQ ID NO: 46 - protein, 5 aa, synthetic construct
  REGION 1..5: note = CDRH1
SYAMS

SEQ ID NO: 47 - protein, 17 aa, synthetic construct
  REGION 1..17: note = CDRH2
AISGSSGSTYYADSVKG

SEQ ID NO: 48 - protein, 8 aa, synthetic construct
  REGION 1..8: note = CDRH3
AQGTSADF

SEQ ID NO: 49 - protein, 5 aa, synthetic construct
  REGION 1..5: note = CDRH1
SYAMS

SEQ ID NO: 50 - protein, 17 aa, synthetic construct
  REGION 1..17: note = CDRH2
AIRSSGGTTYYADSVKG

SEQ ID NO: 51 - protein, 8 aa, synthetic construct
  REGION 1..8: note = CDRH3
SQSTVADY

SEQ ID NO: 52 - protein, 5 aa, synthetic construct
  REGION 1..5: note = CDRH1
SYAMH

SEQ ID NO: 53 - protein, 17 aa, synthetic construct
  REGION 1..17: note = CDRH2
AISSSGGTKYYADSVKG

SEQ ID NO: 54 - protein, 11 aa, synthetic construct
  REGION 1..11: note = CDRH3
GLQGGAGAFDI

SEQ ID NO: 55 - protein, 5 aa, synthetic construct
  REGION 1..5: note = CDRH1
SYAMS

SEQ ID NO: 56 - protein, 17 aa, synthetic construct
  REGION 1..17: note = CDRH2
SISSSSGTTHYADSVKG

SEQ ID NO: 57 - protein, 6 aa, synthetic construct
  REGION 1..6: note = CDRH3
GGAFDY

SEQ ID NO: 58 - protein, 5 aa, synthetic construct
  REGION 1..5: note = CDRH1
SYGMH

SEQ ID NO: 59 - protein, 17 aa, synthetic construct
  REGION 1..17: note = CDRH2
GISSSGGSKYYADSVKG

SEQ ID NO: 60 - protein, 8 aa, synthetic construct
  REGION 1..8: note = CDRH3
HGHQQMDF

SEQ ID NO: 61 - protein, 107 aa, synthetic construct
  REGION 1..107: note = VL
DIQMTQSPSSLSASVGDRVTITCRASQSISRWLNWYQQKPGKAPKLLIYATSTLQSGVPSRFSGSGSGTDFTLTISSLQPEDFATYYCQQSYSFPWTFGQGTKVEIK

SEQ ID NO: 62 - protein, 107 aa, synthetic construct
  REGION 1..107: note = VL
DIQMTQSPSSLSASVGDRVTITCRASQDISNYLNWYQQKPGKAPKLLIYAASSLQSGVPSRFSGSGSGTDFTLTISSLQPEDFATYYCQQSYSFPYTFGQGTKVEIK

SEQ ID NO: 63 - protein, 107 aa, synthetic construct
  REGION 1..107: note = VL
DIQMTQSPSSLSASVGDRVTITCRASQSISRYLNWYQQKPGKAPKLLIYAASSLQSGVPSRFSGSGSGTDFTLTISSLQPEDFATYYCQQSSSTPWTFGQGTKVEIK

SEQ ID NO: 64 - protein, 107 aa, synthetic construct
  REGION 1..107: note = VL
DIQMTQSPSSLSASVGDRVTITCRASQDISSWLNWYQQKPGKAPKLLIYAASRLQSGVPSRFSGSGSGTDFTLTISSLQPEDFATYYCQQAYSFPWTFGQGTKVEIK

SEQ ID NO: 65 - protein, 107 aa, synthetic construct
  REGION 1..107: note = VL
DIQMTQSPSSLSASVGDRVTITCRASQSISNWLNWYQQKPGKAPKLLIYATSRLQSGVPSRFSGSGSGTDFTLTISSLQPEDFATYYCQQSYSFPYTFGQGTKVEIK

SEQ ID NO: 66 - protein, 107 aa, synthetic construct
  REGION 1..107: note = VL
DIQMTQSPSSLSASVGDRVTITCRASQSISRWLNWYQQKPGKAPKLLIYAASRLQSGVPSRFSGSGSGTDFTLTISSLQPEDFATYYCQQSYSTPWTFGQGTKVEIK

SEQ ID NO: 67 - protein, 107 aa, synthetic construct
  REGION 1..107: note = VL
DIQMTQSPSSLSASVGDRVTITCRASQSISNWLNWYQQKPGKAPKLLIYATSRLQSGVPSRFSGSGSGTDFTLTISSLQPEDFATYYCQQSYSFPLTFGQGTKVEIK

SEQ ID NO: 68 - protein, 107 aa, synthetic construct
  REGION 1..107: note = VL
DIQMTQSPSSLSASVGDRVTITCRASQSISNYLNWYQQKPGKAPKLLIYATSTLHSGVPSRFSGSGSGTDFTLTISSLQPEDFATYYCQQSYSFPWTFGQGTKVEIK

SEQ ID NO: 69 - protein, 107 aa, synthetic construct
  REGION 1..107: note = VL
DIQMTQSPSSLSASVGDRVTITCRASQDISRWLNWYQQKPGKAPKLLIYAASTLQSGVPSRFSGSGSGTDFTLTISSLQPEDFATYYCQQSYSFPLTFGQGTKVEIK

SEQ ID NO: 70 - protein, 107 aa, synthetic construct
  REGION 1..107: note = VL
DIQMTQSPSSLSASVGDRVTITCRASQSISSWLNWYQQKPGKAPKLLIYAASRLQSGVPSRFSGSGSGTDFTLTISSLQPEDFATYYCQQTYSFPWTFGQGTKVEIK

SEQ ID NO: 71 - protein, 117 aa, synthetic construct
  REGION 1..117: note = VH
EVQLVESGGGLVQPGGSLRLSCAASGFTFSSYGMSWVRQAPGKGLEWVSAIKGSGGSTYYADSVKGRFTISRDNSKNTLYLQMNSLRAEDTAVYYCAKTYGGEIDYWGQGTLVTVSS

SEQ ID NO: 72 - protein, 117 aa, synthetic construct
  REGION 1..117: note = VH
EVQLVESGGGLVQPGGSLRLSCAASGFTFSDYAMSWVRQAPGKGLEWVSGISSSGGTIYYADSVKGRFTISRDNSKNTLYLQMNSLRAEDTAVYYCAKAIGSWADIWGQGTLVTVSS

SEQ ID NO: 73 - protein, 117 aa, synthetic construct
  REGION 1..117: note = VH
EVQLVESGGGLVQPGGSLRLSCAASGFTFSSYAMHWVRQAPGKGLEWVSAISSSSGTIYYADSVKGRFTISRDNSKNTLYLQMNSLRAEDTAVYYCAKDFGAVFDYWGQGTLVTVSS

SEQ ID NO: 74 - protein, 117 aa, synthetic construct
  REGION 1..117: note = VH
EVQLVESGGGLAQPGGSLRLSCAASGFTFSSYAMHWVRQAPGKGLEWVSSIKSSGGSKNYADSVKGRFTISRDNSKNTLYLQMNSLRAEDTAVYYCAKGYGASFDFWGQGTLVTVSS

SEQ ID NO: 75 - protein, 116 aa, synthetic construct
  REGION 1..116: note = VH
EVQLVESGGGLVQPGGSLRLSCAASGFTFSSYAMHWVRQAPGKGLEWVSAISSSGGSIYYADSVKGRFTISRDNSKNTLYLQMNSLRAEDTAVYYCAKQGLSFDIWGQGTLVTVSS

SEQ ID NO: 76 - protein, 117 aa, synthetic construct
  REGION 1..117: note = VH
EVQLVESGGGLVQPGGSLRLSCAASGFTFSSYAMSWVRQAPGKGLEWVSAISGSSGSTYYADSVKGRFTISRDNSKNTLYLQMNSLRAEDTAVYYCAKAQGTSADFWGQGTLVTVSS

SEQ ID NO: 77 - protein, 117 aa, synthetic construct
  REGION 1..117: note = VH
EVQLVESGGGLVQPGGSLRLSCAASGFTFSSYAMSWVRQAPGKGLEWVSAIRSSGGTTYYADSVKGRFTISRDNSKNTLYLQMNSLRAEDTAVYYCAKSQSTVADYWGQGTLVTVSS

SEQ ID NO: 78 - protein, 120 aa, synthetic construct
  REGION 1..120: note = VH
EVQLVESGGGLVQPGGSLRLSCAASGFTFSSYAMHWVRQAPGKGLEWVSAISSSGGTKYYADSVKGRFTISRDNSKNTLYLQMNSLRAEDTAVYYCAKGLQGGAGAFDIWGQGTLVTVSS

SEQ ID NO: 79 - protein, 115 aa, synthetic construct
  REGION 1..115: note = VH
EVQLVESGGGLVQPGGSLRLSCAASGFTFSSYAMSWVRQAPGKGLEWVSSISSSSGTTHYADSVKGRFTISRDNSKNTLYLQMNSLRAEDTAVYYCAKGGAFDYWGQGTLVTVSS

SEQ ID NO: 80 - protein, 117 aa, synthetic construct
  REGION 1..117: note = VH
EVQLVESGGGLVQPGGSLRLSCAASGFTFSSYGMHWVRQAPGKGLEWVSGISSSGGSKYYADSVKGRFTISRDNSKNTLYLQMNSLRAEDTAVYYCAKHGHQQMDFWGQGTLVTVSS

SEQ ID NO: 81 - DNA, 33 bp, synthetic construct
  misc_feature 1..33: note = CDRL1
  source 1..33: mol_type = other DNA
cgcgctagccagtctatctctcgttggctgaac

SEQ ID NO: 82 - DNA, 21 bp, synthetic construct
  misc_feature 1..21: note = CDRL2
  source 1..21: mol_type = other DNA
gcaacttccactctgcagtct

SEQ ID NO: 83 - DNA, 27 bp, synthetic construct
  misc_feature 1..27: note = CDRL3
  source 1..27: mol_type = other DNA
cagcaatcttactcttttccgtggacg

SEQ ID NO: 84 - DNA, 33 bp, synthetic construct
  misc_feature 1..33: note = CDRL1
  source 1..33: mol_type = other DNA
cgcgctagccaggatatctctaattacctgaac

SEQ ID NO: 85 - DNA, 21 bp, synthetic construct
  misc_feature 1..21: note = CDRL2
  source 1..21: mol_type = other DNA
gcagcatcctctctgcagtct

SEQ ID NO: 86 - DNA, 27 bp, synthetic construct
  misc_feature 1..27: note = CDRL3
  source 1..27: mol_type = other DNA
cagcaatcttactcttttccgtacacg

SEQ ID NO: 87 - DNA, 33 bp, synthetic construct
  misc_feature 1..33: note = CDRL1
  source 1..33: mol_type = other DNA
cgcgctagccagtctatctctcgttacctgaac

SEQ ID NO: 88 - DNA, 21 bp, synthetic construct
  misc_feature 1..21: note = CDRL2
  source 1..21: mol_type = other DNA
gcagcatcctctctgcagtct

SEQ ID NO: 89 - DNA, 27 bp, synthetic construct
  misc_feature 1..27: note = CDRL3
  source 1..27: mol_type = other DNA
cagcaatcttcttctactccgtggacg

SEQ ID NO: 90 - DNA, 33 bp, synthetic construct
  misc_feature 1..33: note = CDRL1
  source 1..33: mol_type = other DNA
cgcgctagccaggatatctcttcttggctgaac

SEQ ID NO: 91 - DNA, 21 bp, synthetic construct
  misc_feature 1..21: note = CDRL2
  source 1..21: mol_type = other DNA
gcagcatcccgtctgcagtct

SEQ ID NO: 92 - DNA, 27 bp, synthetic construct
  misc_feature 1..27: note = CDRL3
  source 1..27: mol_type = other DNA
cagcaagcatactcttttccgtggacg

SEQ ID NO: 93 - DNA, 33 bp, synthetic construct
  misc_feature 1..33: note = CDRL1
  source 1..33: mol_type = other DNA
cgcgctagccagtctatctctaattggctgaac

SEQ ID NO: 94 - DNA, 21 bp, synthetic construct
  misc_feature 1..21: note = CDRL2
  source 1..21: mol_type = other DNA
gcaacttcccgtctgcagtct

SEQ ID NO: 95 - DNA, 27 bp, synthetic construct
  misc_feature 1..27: note = CDRL3
  source 1..27: mol_type = other DNA
cagcaatcttactcttttccgtacacg

SEQ ID NO: 96 - DNA, 33 bp, synthetic construct; identical to SEQ ID NO: 81
  misc_feature 1..33: note = CDRL1
  source 1..33: mol_type = other DNA

SEQ ID NO: 97 - DNA, 21 bp, synthetic construct
  misc_feature 1..21: note = CDRL2
  source 1..21: mol_type = other DNA
gcagcatcccgtctgcagtct

SEQ ID NO: 98 - DNA, 27 bp, synthetic construct
  misc_feature 1..27: note = CDRL3
  source 1..27: mol_type = other DNA
cagcaatcttactctactccgtggacg

SEQ ID NO: 99 - DNA, 33 bp, synthetic construct; identical to SEQ ID NO: 93
  misc_feature 1..33: note = CDRL1
  source 1..33: mol_type = other DNA

SEQ ID NO: 100 - DNA, 21 bp, synthetic construct
  misc_feature 1..21: note = CDRL2
  source 1..21: mol_type = other DNA
gcaacttcccgtctgcagtct

SEQ ID NO: 101 - DNA, 27 bp, synthetic construct
  misc_feature 1..27: note = CDRL3
  source 1..27: mol_type = other DNA
cagcaatcttactcttttccgctgacg

SEQ ID NO: 102 - DNA, 33 bp, synthetic construct
  misc_feature 1..33: note = CDRL1
  source 1..33: mol_type = other DNA
cgcgctagccagtctatctctaattacctgaac

SEQ ID NO: 103 - DNA, 21 bp, synthetic construct
  misc_feature 1..21: note = CDRL2
  source 1..21: mol_type = other DNA
gcaacttccactctgcactct

SEQ ID NO: 104 - DNA, 27 bp, synthetic construct
  misc_feature 1..27: note = CDRL3
  source 1..27: mol_type = other DNA
cagcaatcttactcttttccgtggacg

SEQ ID NO: 105 - DNA, 33 bp, synthetic construct
  misc_feature 1..33: note = CDRL1
  source 1..33: mol_type = other DNA
cgcgctagccaggatatctctcgttggctgaac

SEQ ID NO: 106 - DNA, 21 bp, synthetic construct
  misc_feature 1..21: note = CDRL2
  source 1..21: mol_type = other DNA
gcagcatccactctgcagtct

SEQ ID NO: 107 - DNA, 27 bp, synthetic construct
  misc_feature 1..27: note = CDRL3
  source 1..27: mol_type = other DNA
cagcaatcttactcttttccgctgacg

SEQ ID NO: 108 - DNA, 33 bp, synthetic construct
  misc_feature 1..33: note = CDRL1
  source 1..33: mol_type = other DNA
cgcgctagccagtctatctcttcttggctgaac

SEQ ID NO: 109 - DNA, 21 bp, synthetic construct
  misc_feature 1..21: note = CDRL2
  source 1..21: mol_type = other DNA
gcagcatcccgtctgcagtct

SEQ ID NO: 110 - DNA, 27 bp, synthetic construct
  misc_feature 1..27: note = CDRL3
  source 1..27: mol_type = other DNA
cagcaaacttactcttttccgtggacg

SEQ ID NO: 111 - DNA, 15 bp, synthetic construct
  misc_feature 1..15: note = CDRH1
  source 1..15: mol_type = other DNA
tcttatggtatgtct

SEQ ID NO: 112 - DNA, 51 bp, synthetic construct
  misc_feature 1..51: note = CDRH2
  source 1..51: mol_type = other DNA
gcaatcaaaggttctggtggttctacttactatgccgattcagtgaagggt

SEQ ID NO: 113 - DNA, 24 bp, synthetic construct
  misc_feature 1..24: note = CDRH3
  source 1..24: mol_type = other DNA
acttacggtggtgaaatcgattac

SEQ ID NO: 114 - DNA, 15 bp, synthetic construct
  misc_feature 1..15: note = CDRH1
  source 1..15: mol_type = other DNA
gattatgcaatgtct

SEQ ID NO: 115 - DNA, 51 bp, synthetic construct
  misc_feature 1..51: note = CDRH2
  source 1..51: mol_type = other DNA
ggtatctcttcttctggtggtactatctactatgccgattcagtgaagggt

SEQ ID NO: 116 - DNA, 24 bp, synthetic construct
  misc_feature 1..24: note = CDRH3
  source 1..24: mol_type = other DNA
gcaatcggttcttgggcagatatc

SEQ ID NO: 117 - DNA, 15 bp, synthetic construct
  misc_feature 1..15: note = CDRH1
  source 1..15: mol_type = other DNA
tcttatgcaatgcac

SEQ ID NO: 118 - DNA, 51 bp, synthetic construct
  misc_feature 1..51: note = CDRH2
  source 1..51: mol_type = other DNA
gcaatctcttcttcttctggtactatctactatgccgattcagtgaagggt

SEQ ID NO: 119 - DNA, 24 bp, synthetic construct
  misc_feature 1..24: note = CDRH3
  source 1..24: mol_type = other DNA
gatttcggtgcagttttcgattac

SEQ ID NO: 120 - DNA, 15 bp, synthetic construct
  misc_feature 1..15: note = CDRH1
  source 1..15: mol_type = other DNA
tcttatgcaatgcac

SEQ ID NO: 121 - DNA, 51 bp, synthetic construct
  misc_feature 1..51: note = CDRH2
  source 1..51: mol_type = other DNA
tctatcaaatcttctggtggttctaaaaattatgccgattcagtgaagggt

SEQ ID NO: 122 - DNA, 24 bp, synthetic construct
  misc_feature 1..24: note = CDRH3
  source 1..24: mol_type = other DNA
ggttacggtgcatctttcgatttc

SEQ ID NO: 123 - DNA, 15 bp, synthetic construct
  misc_feature 1..15: note = CDRH1
  source 1..15: mol_type = other DNA
tcttatgcaatgcac

SEQ ID NO: 124 - DNA, 51 bp, synthetic construct
  misc_feature 1..51: note = CDRH2
  source 1..51: mol_type = other DNA
gcaatctcttcttctggtggttctatctactatgccgattcagtgaagggt

SEQ ID NO: 125 - DNA, 21 bp, synthetic construct
  misc_feature 1..21: note = CDRH3
  source 1..21: mol_type = other DNA
cagggtctgtctttcgatatc

SEQ ID NO: 126 - DNA, 15 bp, synthetic construct
  misc_feature 1..15: note = CDRH1
  source 1..15: mol_type = other DNA
tcttatgcaatgtct

SEQ ID NO: 127 - DNA, 51 bp, synthetic construct
  misc_feature 1..51: note = CDRH2
  source 1..51: mol_type = other DNA
gcaatctctggttcttctggttctacttactatgccgattcagtgaagggt

SEQ ID NO: 128 - DNA, 24 bp, synthetic construct
  misc_feature 1..24: note = CDRH3
  source 1..24: mol_type = other DNA
gcacagggtacttctgcagatttc

SEQ ID NO: 129 - DNA, 15 bp, synthetic construct
  misc_feature 1..15: note = CDRH1
  source 1..15: mol_type = other DNA
tcttatgcaatgtct

SEQ ID NO: 130 - DNA, 51 bp, synthetic construct
  misc_feature 1..51: note = CDRH2
  source 1..51: mol_type = other DNA
gcaatccgttcttctggtggtactacttactatgccgattcagtgaagggt

SEQ ID NO: 131 - DNA, 24 bp, synthetic construct
  misc_feature 1..24: note = CDRH3
  source 1..24: mol_type = other DNA
tctcagtctactgttgcagattac

SEQ ID NO: 132 - DNA, 15 bp, synthetic construct
  misc_feature 1..15: note = CDRH1
  source 1..15: mol_type = other DNA
tcttatgcaatgcac

SEQ ID NO: 133 - DNA, 51 bp, synthetic construct
  misc_feature 1..51: note = CDRH2
  source 1..51: mol_type = other DNA
gcaatctcttcttctggtggtactaaatactatgccgattcagtgaagggt

SEQ ID NO: 134 - DNA, 33 bp, synthetic construct
  misc_feature 1..33: note = CDRH3
  source 1..33: mol_type = other DNA
ggtctgcagggtggtgcaggtgcatttgatatc

SEQ ID NO: 135 - DNA, 15 bp, synthetic construct
  misc_feature 1..15: note = CDRH1
  source 1..15: mol_type = other DNA
tcttatgcaatgtct

SEQ ID NO: 136 - DNA, 51 bp, synthetic construct
  misc_feature 1..51: note = CDRH2
  source 1..51: mol_type = other DNA
tctatctcttcttcttctggtactactcactatgccgattcagtgaagggt

SEQ ID NO: 137 - DNA, 18 bp, synthetic construct
  misc_feature 1..18: note = CDRH3
  source 1..18: mol_type = other DNA
ggtggtgcattcgattac

SEQ ID NO: 138 - DNA, 15 bp, synthetic construct
  misc_feature 1..15: note = CDRH1
  source 1..15: mol_type = other DNA
tcttatggtatgcac

SEQ ID NO: 139 - DNA, 51 bp, synthetic construct
  misc_feature 1..51: note = CDRH2
  source 1..51: mol_type = other DNA
ggtatctcttcttctggtggttctaaatactatgccgattcagtgaagggt

SEQ ID NO: 140 - DNA, 24 bp, synthetic construct
  misc_feature 1..24: note = CDRH3
  source 1..24: mol_type = other DNA
catggtcatcagcagatggatttc

SEQ ID NO: 141 - DNA, 321 bp, synthetic construct
  misc_feature 1..321: note = VL
  source 1..321: mol_type = other DNA
gacattcaaatgacgcagagtccctcctcactgagtgctagcgtgggcgatcgtgtgacaattacttgtcgcgctagccagtctatctctcgttggctgaactggtatcagcagaaaccgggcaaggcgccaaaattgctgatttacgcaacttccactctgcagtctggtgtaccgtcccgtttctctggcagcggttctggtacggattttaccctgaccatctcaagcctccagcctgaagattttgccacctattattgtcagcaatcttactcttttccgtggacgttcgggcagggaactaaagtggaaattaaa

SEQ ID NO: 142 - DNA, 321 bp, synthetic construct
  misc_feature 1..321: note = VL
  source 1..321: mol_type = other DNA
gacattcaaatgacgcagagtccctcctcactgagtgctagcgtgggcgatcgtgtgacaattacttgtcgcgctagccaggatatctctaattacctgaactggtatcagcagaaaccgggcaaggcgccaaaattgctgatttacgcagcatcctctctgcagtctggtgtaccgtcccgtttctctggcagcggttctggtacggattttaccctgaccatctcaagcctccagcctgaagattttgccacctattattgtcagcaatcttactcttttccgtacacgttcgggcagggaactaaagtggaaattaaa

SEQ ID NO: 143 - DNA, 321 bp, synthetic construct
  misc_feature 1..321: note = VL
  source 1..321: mol_type = other DNA
gacattcaaatgacgcagagtccctcctcactgagtgctagcgtgggcgatcgtgtgacaattacttgtcgcgctagccagtctatctctcgttacctgaactggtatcagcagaaaccgggcaaggcgccaaaattgctgatttacgcagcatcctctctgcagtctggtgtaccgtcccgtttctctggcagcggttctggtacggattttaccctgaccatctcaagcctccagcctgaagattttgccacctattattgtcagcaatcttcttctactccgtggacgttcgggcagggaactaaagtggaaattaaa

SEQ ID NO: 144 - DNA, 321 bp, synthetic construct
  misc_feature 1..321: note = VL
  source 1..321: mol_type = other DNA
gacattcaaatgacgcagagtccctcctcactgagtgctagcgtgggcgatcgtgtgacaattacttgtcgcgctagccaggatatctcttcttggctgaactggtatcagcagaaaccgggcaaggcgccaaaattgctgatttacgcagcatcccgtctgcagtctggtgtaccgtcccgtttctctggcagcggttctggtacggattttaccctgaccatctcaagcctccagcctgaagattttgccacctattattgtcagcaagcatactcttttccgtggacgttcgggcagggaactaaagtggaaattaaa

SEQ ID NO: 145 - DNA, 321 bp, synthetic construct
  misc_feature 1..321: note = VL
  source 1..321: mol_type = other DNA
gacattcaaatgacgcagagtccctcctcactgagtgctagcgtgggcgatcgtgtgacaattacttgtcgcgctagccagtctatctctaattggctgaactggtatcagcagaaaccgggcaaggcgccaaaattgctgatttacgcaacttcccgtctgcagtctggtgtaccgtcccgtttctctggcagcggttctggtacggattttaccctgaccatctcaagcctccagcctgaagattttgccacctattattgtcagcaatcttactcttttccgtacacgttcgggcagggaactaaagtggaaattaaa

SEQ ID NO: 146 - DNA, 321 bp, synthetic construct
  misc_feature 1..321: note = VL
  source 1..321: mol_type = other DNA
gacattcaaatgacgcagagtccctcctcactgagtgctagcgtgggcgatcgtgtgacaattacttgtcgcgctagccagtctatctctcgttggctgaactggtatcagcagaaaccgggcaaggcgccaaaattgctgatttacgcagcatcccgtctgcagtctggtgtaccgtcccgtttctctggcagcggttctggtacggattttaccctgaccatctcaagcctccagcctgaagattttgccacctattattgtcagcaatcttactctactccgtggacgttcgggcagggaactaaagtggaaattaaa

SEQ ID NO: 147 - DNA, 321 bp, synthetic construct
  misc_feature 1..321: note = VL
  source 1..321: mol_type = other DNA
gacattcaaatgacgcagagtccctcctcactgagtgctagcgtgggcgatcgtgtgacaattacttgtcgcgctagccagtctatctctaattggctgaactggtatcagcagaaaccgggcaaggcgccaaaattgctgatttacgcaacttcccgtctgcagtctggtgtaccgtcccgtttctctggcagcggttctggtacggattttaccctgaccatctcaagcctccagcctgaagattttgccacctattattgtcagcaatcttactcttttccgctgacgttcgggcagggaactaaagtggaaattaaa

SEQ ID NO: 148 - DNA, 321 bp, synthetic construct
  misc_feature 1..321: note = VL
  source 1..321: mol_type = other DNA
gacattcaaatgacgcagagtccctcctcactgagtgctagcgtgggcgatcgtgtgacaattacttgtcgcgctagccagtctatctctaattacctgaactggtatcagcagaaaccgggcaaggcgccaaaattgctgatttacgcaacttccactctgcactctggtgtaccgtcccgtttctctggcagcggttctggtacggattttaccctgaccatctcaagcctccagcctgaagattttgccacctattattgtcagcaatcttactcttttccgtggacgttcgggcagggaactaaagtggaaattaaa

SEQ ID NO: 149 - DNA, 321 bp, synthetic construct
  misc_feature 1..321: note = VL
  source 1..321: mol_type = other DNA
gacattcaaatgacgcagagtccctcctcactgagtgctagcgtgggcgatcgtgtgacaattacttgtcgcgctagccaggatatctctcgttggctgaactggtatcagcagaaaccgggcaaggcgccaaaattgctgatttacgcagcatccactctgcagtctggtgtaccgtcccgtttctctggcagcggttctggtacggattttaccctgaccatctcaagcctccagcctgaagattttgccacctattattgtcagcaatcttactcttttccgctgacgttcgggcagggaactaaagtggaaattaaa

SEQ ID NO: 150 - DNA, 321 bp, synthetic construct
  misc_feature 1..321: note = VL
  source 1..321: mol_type = other DNA
gacattcaaatgacgcagagtccctcctcactgagtgctagcgtgggcgatcgtgtgacaattacttgtcgcgctagccagtctatctcttcttggctgaactggtatcagcagaaaccgggcaaggcgccaaaattgctgatttacgcagcatcccgtctgcagtctggtgtaccgtcccgtttctctggcagcggttctggtacggattttaccctgaccatctcaagcctccagcctgaagattttgccacctattattgtcagcaaacttactcttttccgtggacgttcgggcagggaactaaagtggaaattaaa

SEQ ID NO: 151 - DNA, 351 bp, synthetic construct
  misc_feature 1..351: note = VH
  source 1..351: mol_type = other DNA
gaagtacagttggtcgaaagtggcggtggcctcgtgcaaccgggtggttcactgcgtctgagctgcgccgcctcgggttttactttctcttcttatggtatgtcttgggttcgtcaggcgccgggcaagggtctcgaatgggtttcagcaatcaaaggttctggtggttctacttactatgccgattcagtgaagggtcgctttaccatttcccgtgacaactctaagaatactctgtatctgcagatgaactcgctgcgtgccgaagacacggccgtctattattgcgccaaaacttacggtggtgaaatcgattactggggtcagggcactttagtgaccgtctcatcg

SEQ ID NO: 152 - DNA, 351 bp, synthetic construct
  misc_feature 1..351: note = VH
  source 1..351: mol_type = other DNA
gaagtacagttggtcgaaagtggcggtggcctcgtgcaaccgggtggttcactgcgtctgagctgcgccgcctcgggttttactttctctgattatgcaatgtcttgggttcgtcaggcgccgggcaagggtctcgaatgggtttcaggtatctcttcttctggtggtactatctactatgccgattcagtgaagggtcgctttaccatttcccgtgacaactctaagaatactctgtatctgcagatgaactcgctgcgtgccgaagacacggccgtctattattgcgccaaagcaatcggttcttgggcagatatctggggtcagggcactttagtgaccgtctcatcg

SEQ ID NO: 153 - DNA, 351 bp, synthetic construct
  misc_feature 1..351: note = VH
  source 1..351: mol_type = other DNA
gaagtacagttggtcgaaagtggcggtggcctcgtgcaaccgggtggttcactgcgtctgagctgcgccgcctcgggttttactttctcttcttatgcaatgcactgggttcgtcaggcgccgggcaagggtctcgaatgggtttcagcaatctcttcttcttctggtactatctactatgccgattcagtgaagggtcgctttaccatttcccgtgacaactctaagaatactctgtatctgcagatgaactcgctgcgtgccgaagacacggccgtctattattgcgccaaagatttcggtgcagttttcgattactggggtcagggcactttagtgaccgtctcatcg

SEQ ID NO: 154 - DNA, 351 bp, synthetic construct
  misc_feature 1..351: note = VH
  source 1..351: mol_type = other DNA
gaagtacagttggtcgaaagtggcggtggcctcgcgcaaccgggtggttcactgcgtctgagctgcgccgcctcgggttttactttctcttcttatgcaatgcactgggttcgtcaggcgccgggcaagggtctcgaatgggtttcatctatcaaatcttctggtggttctaaaaattatgccgattcagtgaagggtcgctttaccatttcccgtgacaactctaagaatactctgtatctgcagatgaactcgctgcgtgccgaagacacggccgtctattattgcgccaaaggttacggtgcatctttcgatttctggggtcagggcactttagtgaccgtctcatcg

SEQ ID NO: 155 - DNA, 348 bp, synthetic construct
  misc_feature 1..348: note = VH
  source 1..348: mol_type = other DNA
gaagtacagttggtcgaaagtggcggtggcctcgtgcaaccgggtggttcactgcgtctgagctgcgccgcctcgggttttactttctcttcttatgcaatgcactgggttcgtcaggcgccgggcaagggtctcgaatgggtttcagcaatctcttcttctggtggttctatctactatgccgattcagtgaagggtcgctttaccatttcccgtgacaactctaagaatactctgtatctgcagatgaactcgctgcgtgccgaagacacggccgtctattattgcgccaaacagggtctgtctttcgatatctggggtcagggcactttagtgaccgtctcatcg

SEQ ID NO: 156 - DNA, 351 bp, synthetic construct
  misc_feature 1..351: note = VH
  source 1..351: mol_type = other DNA
gaagtacagttggtcgaaagtggcggtggcctcgtgcaaccgggtggttcactgcgtctgagctgcgccgcctcgggttttactttctcttcttatgcaatgtcttgggttcgtcaggcgccgggcaagggtctcgaatgggtttcagcaatctctggttcttctggttctacttactatgccgattcagtgaagggtcgctttaccatttcccgtgacaactctaagaatactctgtatctgcagatgaactcgctgcgtgccgaagacacggccgtctattattgcgccaaagcacagggtacttctgcagatttctggggtcagggcactttagtgaccgtctcatcg

SEQ ID NO: 157 - DNA, 351 bp, synthetic construct
  misc_feature 1..351: note = VH
  source 1..351: mol_type = other DNA
gaagtacagttggtcgaaagtggcggtggcctcgtgcaaccgggtggttcactgcgtctgagctgcgccgcctcgggttttactttctcttcttatgcaatgtcttgggttcgtcaggcgccgggcaagggtctcgaatgggtttcagcaatccgttcttctggtggtactacttactatgccgattcagtgaagggtcgctttaccatttcccgtgacaactctaagaatactctgtatctgcagatgaactcgctgcgtgccgaagacacggccgtctattattgcgccaaatctcagtctactgttgcagattactggggtcagggcactttagtgaccgtctcatcg

SEQ ID NO: 158 - DNA, 360 bp, synthetic construct
  misc_feature 1..360: note = VH
  source 1..360: mol_type = other DNA
gaagtacagttggtcgaaagtggcggtggcctcgtgcaaccgggtggttcactgcgtctgagctgcgccgcctcgggttttactttctcttcttatgcaatgcactgggttcgtcaggcgccgggcaagggtctcgaatgggtttcagcaatctcttcttctggtggtactaaatactatgccgattcagtgaagggtcgctttaccatttcccgtgacaactctaagaatactctgtatctgcagatgaactcgctgcgtgccgaagacacggccgtctattattgcgccaaaggtctgcagggtggtgcaggtgcatttgatatctggggtcagggtactctggttactgtatcatcg

SEQ ID NO: 159 - DNA, 345 bp, synthetic construct
  misc_feature 1..345: note = VH
  source 1..345: mol_type = other DNA
gaagtacagttggtcgaaagtggcggtggcctcgtgcaaccgggtggttcactgcgtctgagctgcgccgcctcgggttttactttctcttcttatgcaatgtcttgggttcgtcaggcgccgggcaagggtctcgaatgggtttcatctatctcttcttcttctggtactactcactatgccgattcagtgaagggtcgctttaccatttcccgtgacaactctaagaatactctgtatctgcagatgaactcgctgcgtgccgaagacacggccgtctattattgcgccaaaggtggtgcattcgattactggggtcagggcactttagtgaccgtctcatcg

SEQ ID NO: 160 - DNA, 351 bp, synthetic construct
  misc_feature 1..351: note = VH
  source 1..351: mol_type = other DNA
gaagtacagttggtcgaaagtggcggtggcctcgtgcaaccgggtggttcactgcgtctgagctgcgccgcctcgggttttactttctcttcttatggtatgcactgggttcgtcaggcgccgggcaagggtctcgaatgggtttcaggtatctcttcttctggtggttctaaatactatgccgattcagtgaagggtcgctttaccatttcccgtgacaactctaagaatactctgtatctgcagatgaactcgctgcgtgccgaagacacggccgtctattattgcgccaaacatggtcatcagcagatggatttctggggtcagggcactttagtgaccgtctcatcg